European Patent Application EP 4 445 912 A1, published October 16, 2024. Title: P329G antibody targeting BCMA, combination with chimeric antigen receptor cells and use thereof. Applicant: INNOVENT CELLS PHARMACEUTICALS (SU ZHOU) CO., LTD. Application WO. The sequence listing filed with the application follows.

SEQUENCE LISTING (41 sequences)

SEQ ID NO: 1 - protein, 452 aa, artificial sequence
MALPVTALLLPLALLLHAARPEVQLVESGGGLVQPGGSLRLSCAASGFTFSRYWMNWVRQAPGKGLEWVGEITPDSSTINYAPSLKGRFTISRDNAKNSLYLQMNSLRAEDTAVYYCARPYDYGAWFASWGQGTLVTVSSGGGGSGGGGSGGGGSGGGGSQAVVTQEPSLTVSPGGTVTLTCRSSTGAVTTSNYANWVQEKPDHLFTGLIGGTNKRAPGTPARFSGSLLGGKAALTLSGAQPEDEAEYYCALWYSNHWVFGGGTKLTVLGGGGSIYIWAPLAGTCGVLLLSLVITLYCKRGRKKLLYIFKQPFMRPVQTTQEEDGCSCRFPEEEEGGCELRVKFSRSADAPAYQQGQNQLYNELNLGRREEYDVLDKRRGRDPEMGGKPRRKNPQEGLYNELQKDKMAEAYSEIGMKGERRRGKGHDGLYQGLSTATKDTYDALHMQALPPR

SEQ ID NO: 2 - protein, 119 aa, artificial sequence
QLQLQESGPGLVKPSETLSLTCTVSGGSIVSSSYYWTWIRQPPGKGLEWIGSISIAGSTYYNPSLKSRVTISVDTSKNQFSLKLSSVTAADTAVYYCARDRGDQILDVWSQGTMVTVSS

SEQ ID NO: 3 - protein, 106 aa, artificial sequence
DIQMTQSPSSLSASVGDRVTITCRASQSISRYLNWYQQKPGKAPKLLIYAASSLQSGVPSRFSGSGSGTDFTLTISSLQPEDFATYYCQQKYFDITFGGGTKVEIK

SEQ ID NO: 4 - protein, 330 aa, artificial sequence [sequence omitted]

SEQ ID NO: 5 - protein, 330 aa, artificial sequence
ASTKGPSVFPLAPSSKSTSGGTAALGCLVKDYFPEPVTVSWNSGALTSGVHTFPAVLQSSGLYSLSSVVTVPSSSLGTQTYICNVNHKPSNTKVDKKVEPKSCDKTHTCPPCPAPELLGGPSVFLFPPKPKDTLMISRTPEVTCVVVDVSHEDPEVKFNWYVDGVEVHNAKTKPREEQYNSTYRVVSVLTVLHQDWLNGKEYKCKVSNKALGAPIEKTISKAKGQPREPQVYTLPPSRDELTKNQVSLTCLVKGFYPSDIAVEWESNGQPENNYKTTPPVLDSDGSFFLYSKLTVDKSRWQQGNVFSCSVMHEALHNHYTQKSLSLSPGK

SEQ ID NO: 6 - protein, 107 aa, artificial sequence [sequence omitted]

SEQ ID NO: 7 - protein, 476 aa, artificial sequence
EVQLVESGGGLVQPGGSLRLSCAASGFTFSRYWMNWVRQAPGKGLEWVGEITPDSSTINYAPSLKGRFTISRDNAKNSLYLQMNSLRAEDTAVYYCARPYDYGAWFASWGQGTLVTVSSGGGGSGGGGSGGGGSGGGGSQAVVTQEPSLTVSPGGTVTLTCRSSTGAVTTSNYANWVQEKPDHLFTGLIGGTNKRAPGTPARFSGSLLGGKAALTLSGAQPEDEAEYYCALWYSNHWVFGGGTKLTVLGGGGSSKPTCPPPELLGGPSVFIFPPKPKDTLMISRTPEVTCVVVDVSQDDPEVQFTWYINNEQVRTARPPLREQQFNSTIRVVSTLPIAHQDWLRGKEFKCKVHNKALPAPIEKTISKARGQPLEPKVYTMGPPREELSSRSVSLTCMINGFYPSDISVEWEKNGKAEDNYKTTPAVLDSDGSYFLYSKLSVPTSEWQRGDVFTCSVMHEALHNHYTQKSISRSPGK

SEQ ID NO: 8 - protein, 493 aa, artificial sequence
MALPVTALLLPLALLLHAARPDIVLTQSPPSLAMSLGKRATISCRASESVTILGSHLIHWYQQKPGQPPTLLIQLASNVQTGVPARFSGSGSRTDFTLTIDPVEEDDVAVYYCLQSRTIPRTFGGGTKLEIKGSTSGSGKPGSGEGSTKGQIQLVQSGPELKKPGETVKISCKASGYTFTDYSINWVKRAPGKGLKWMGWINTETREPAYAYDFRGRFAFSLETSASTAYLQINNLKYEDTATYFCALDYSYAMDYWGQGTSVTVSSAAATTTPAPRPPTPAPTIASQPLSLRPEACRPAAGGAVHTRGLDFACDIYIWAPLAGTCGVLLLSLVITLYCKRGRKKLLYIFKQPFMRPVQTTQEEDGCSCRFPEEEEGGCELRVKFSRSADAPAYQQGQNQLYNELNLGRREEYDVLDKRRGRDPEMGGKPRRKNPQEGLYNELQKDKMAEAYSEIGMKGERRRGKGHDGLYQGLSTATKDTYDALHMQALPPR

SEQ ID NO: 9 - protein, 121 aa, artificial sequence
QVQLVQSGAEVKKPGSSVKVSCKASGGTFSNDVISWVRQAPGQGLEWMGVIIPIFGIANYAQKFQGRVTITADESTSTAYMELSSLRSEDTAVYYCARGRGYYSSWLHDIWGQGTMVTVSS

SEQ ID NO: 10 - protein, 106 aa, artificial sequence
DIQMTQSPSSLSASVGDRVTITCQASQDITNYLNWYQQKPGKAPKLLIYDASNLETGVPSRFSGSGSGTDFTFTISSLQPEDIATYYCQQAFDLITFGGGTKVEIK

SEQ ID NO: 11 - protein, 21 aa, artificial sequence
MALPVTALLLPLALLLHAARP

SEQ ID NO: 12 - protein, 119 aa, artificial sequence
EVQLVESGGGLVQPGGSLRLSCAASGFTFSRYWMNWVRQAPGKGLEWVGEITPDSSTINYAPSLKGRFTISRDNAKNSLYLQMNSLRAEDTAVYYCARPYDYGAWFASWGQGTLVTVSS

SEQ ID NO: 13 - protein, 109 aa, artificial sequence
QAVVTQEPSLTVSPGGTVTLTCRSSTGAVTTSNYANWVQEKPDHLFTGLIGGTNKRAPGTPARFSGSLLGGKAALTLSGAQPEDEAEYYCALWYSNHWVFGGGTKLTVL

SEQ ID NO: 14 - protein, 5 aa, artificial sequence
GGGGS

SEQ ID NO: 15 - protein, 24 aa, artificial sequence
IYIWAPLAGTCGVLLLSLVITLYC

SEQ ID NO: 16 - protein, 42 aa, artificial sequence
KRGRKKLLYIFKQPFMRPVQTTQEEDGCSCRFPEEEEGGCEL

SEQ ID NO: 17 - protein, 112 aa, artificial sequence
RVKFSRSADAPAYQQGQNQLYNELNLGRREEYDVLDKRRGRDPEMGGKPRRKNPQEGLYNELQKDKMAEAYSEIGMKGERRRGKGHDGLYQGLSTATKDTYDALHMQALPPR

SEQ ID NO: 18 - protein, 45 aa, artificial sequence
TTTPAPRPPTPAPTIASQPLSLRPEACRPAAGGAVHTRGLDFACD

SEQ ID NO: 19 - protein, 5 aa, artificial sequence
RYWMN

SEQ ID NO: 20 - protein, 17 aa, artificial sequence
EITPDSSTINYAPSLKG

SEQ ID NO: 21 - protein, 10 aa, artificial sequence
PYDYGAWFAS

SEQ ID NO: 22 - protein, 14 aa, artificial sequence
RSSTGAVTTSNYAN

SEQ ID NO: 23 - protein, 7 aa, artificial sequence
GTNKRAP

SEQ ID NO: 24 - protein, 9 aa, artificial sequence
ALWYSNHWV

SEQ ID NO: 25 - protein, 7 aa, artificial sequence
SSSYYWT

SEQ ID NO: 26 - protein, 16 aa, artificial sequence
SISIAGSTYYNPSLKS

SEQ ID NO: 27 - protein, 9 aa, artificial sequence
DRGDQILDV

SEQ ID NO: 28 - protein, 11 aa, artificial sequence
RASQSISRYLN

SEQ ID NO: 29 - protein, 7 aa, artificial sequence
AASSLQS

SEQ ID NO: 30 - protein, 8 aa, artificial sequence
QQKYFDIT

SEQ ID NO: 31 - protein, 5 aa, artificial sequence
NDVIS

SEQ ID NO: 32 - protein, 17 aa, artificial sequence
VIIPIFGIANYAQKFQG

SEQ ID NO: 33 - protein, 12 aa, artificial sequence
GRGYYSSWLHDI

SEQ ID NO: 34 - protein, 11 aa, artificial sequence
QASQDITNYLN

SEQ ID NO: 35 - protein, 7 aa, artificial sequence
DASNLET

SEQ ID NO: 36 - protein, 8 aa, artificial sequence
QQAFDLIT

SEQ ID NO: 37 - protein, 119 aa, artificial sequence
QLQLQESGPGLVKPSETLSLTCTVSGGSISSSSYYWGWIRQPPGKGLEWIGSISYSGSTYYNPSLKSRVTISVDTSKNQFSLKLSSVTAADTAVYYCARDRGDTILDVWGQGTMVTVSS

SEQ ID NO: 38 - protein, 106 aa, artificial sequence; identical to SEQ ID NO: 3

SEQ ID NO: 39 - protein, 121 aa, artificial sequence
QVQLVQSGAEVKKPGSSVKVSCKASGGTFSNYAISWVRQAPGQGLEWMGGIIPIFGTANYAQKFQGRVTITADESTSTAYMELSSLRSEDTAVYYCARGRGYYSSWLFDIWGQGTMVTVSS

SEQ ID NO: 40 - protein, 106 aa, artificial sequence; identical to SEQ ID NO: 10

SEQ ID NO: 41 - protein, 20 aa, artificial sequence
GGGGSGGGGSGGGGSGGGGS